European Patent Specification EP 3 050 961 B1, published June 28, 2023. Title: Methods of improving efficiency of inducing pluripotent stem cells. Applicant: DNAVEC CORPORATION. The sequence listing filed with the application follows.

SEQUENCE LISTING (15 sequences)

SEQ ID NO: 1 - RNA, 10 nt, Artificial sequence
  artificially synthesized sequence
ucccwvuuwc

SEQ ID NO: 2 - RNA, 10 nt, Artificial sequence
  artificially synthesized sequence
ucccaguuuc

SEQ ID NO: 3 - RNA, 10 nt, Artificial sequence
  artificially synthesized sequence
ucccacuuac

SEQ ID NO: 4 - RNA, 10 nt, Artificial sequence
  artificially synthesized sequence
ucccacuuuc

SEQ ID NO: 5 - DNA, 10 bp, Artificial sequence
  artificially synthesized sequence
agggtcaaag

SEQ ID NO: 6 - DNA, 10 bp, Artificial sequence
  artificially synthesized sequence
agggtgaatg

SEQ ID NO: 7 - DNA, 10 bp, Artificial sequence
  artificially synthesized sequence
agggtgaaag

SEQ ID NO: 8 - DNA, 1317 bp, Artificial sequence
  artificially synthesized sequence
  CDS (1)..(1317)
atgcccctcaacgttagcttcaccaacaggaactatgacctcgactacgactcggtgcagccgtatttctactgcgacgaggaggagaacttctaccagcagcagcagcagagcgagctgcagcccccggcgcccagcgaggatatctggaagaaattcgagctgctgcccaccccgcccctgtcccctagccgccgctccgggctctgctcgccctcctacgttgcggtcacacccttctcccttcggggagacaacgacggcggtggcgggagcttctccacggccgaccagctggagatggtgaccgagctgctgggaggagacatggtgaaccagagtttcatctgcgacccggacgacgagaccttcatcaagaacatcatcatccaggactgtatgtggagcggcttctcggccgccgccaagctcgtctcagagaagctggcctcctaccaggctgcgcgcaaagacagcggcagcccgaaccccgcccgcggccacagcgtctgctccacctccagcttgtacctgcaggatctgagcgccgccgcctcagagtgcatcgacccctcggtggtcttcccctaccctctcaacgacagcagctcgcccaagtcctgcgcctcgcaagactccagcgccttctctccgtcctcggattctctgctctcctcgacggagtcctccccgcagggcagccccgagcccctggtgctccatgaggagacaccgcccaccaccagcagcgactctgaggaggaacaagaagatgaggaagaaatcgatgttgtttctgtggaaaagaggcaggctcctggcaaaaggtcagagtctggatcaccttctgctggaggccacagcaaacctcctcacagcccactggtcctcaagaggtgccacgtctccacacatcagcacaactacgcagcgcctccctccactcggaaggactatcctgctgccaagagggtcaagttggacagtgtcagagtcctgagacagatcagcaacaaccgaaaatgcaccagccccaggtcctcggacaccgaggagaatgtcaagaggcgaacacacaacgtcttggagcgccagaggaggaacgagctaaaacggagcttcttcgccctgcgtgaccagatcccggagttggaaaacaatgaaaaggcccccaaggtagttatccttaagaaggccacagcatacatcctgtccgtccaagcagaggagcaaaagctcatttctgaagaggacttgttgcggaaacgacgagaacagttgaaacacaaacttgaacagctacggaactcttgtgcg

SEQ ID NO: 9 - protein, 439 aa, Artificial sequence
  Synthetic Construct
MPLNVSFTNRNYDLDYDSVQPYFYCDEEENFYQQQQQSELQPPAPSEDIWKKFELLPTPPLSPSRRSGLCSPSYVAVTPFSLRGDNDGGGGSFSTADQLEMVTELLGGDMVNQSFICDPDDETFIKNIIIQDCMWSGFSAAAKLVSEKLASYQAARKDSGSPNPARGHSVCSTSSLYLQDLSAAASECIDPSVVFPYPLNDSSSPKSCASQDSSAFSPSSDSLLSSTESSPQGSPEPLVLHEETPPTTSSDSEEEQEDEEEIDVVSVEKRQAPGKRSESGSPSAGGHSKPPHSPLVLKRCHVSTHQHNYAAPPSTRKDYPAAKRVKLDSVRVLRQISNNRKCTSPRSSDTEENVKRRTHNVLERQRRNELKRSFFALRDQIPELENNEKAPKVVILKKATAYILSVQAEEQKLISEEDLLRKRREQLKHKLEQLRNSCA

SEQ ID NO: 10 - DNA, 40 bp, Artificial sequence
  artificially synthesized sequence
gaaatttcacctaagcggccgcaatggcagatatctatag

SEQ ID NO: 11 - DNA, 40 bp, Artificial sequence
  artificially synthesized sequence
ctatagatatctgccattgcggccgcttaggtgaaatttc

SEQ ID NO: 12 - DNA, 22 bp, Artificial sequence
  artificially synthesized sequence
agagaacaagactaaggctacc

SEQ ID NO: 13 - DNA, 21 bp, Artificial sequence
  artificially synthesized sequence
accttgacaatcctgatgtgg

SEQ ID NO: 14 - DNA, 22 bp, Artificial sequence
  artificially synthesized sequence
ccatcaacactccccaaggacc

SEQ ID NO: 15 - DNA, 22 bp, Artificial sequence
  artificially synthesized sequence
agacgtgatgcgtttgaggccc